European Patent Application EP 4 755 915 A1, published June 10, 2026. Title: Antibodies and pharmaceutical compositions containing the same for treating immune diseases. Applicant: MEDYTOX INC. Application KR PT24-5319, filed July 31, 2024. The sequence listing filed with the application follows.

SEQUENCE LISTING (76 sequences)

SEQ ID NO: 1 - protein, 456 aa, synthetic construct
  REGION 1..456: note = mAb637-IgG1 heavy chain
QVQLLESGGGLVKPGGSLRLSCAASGFKSTDYYMAWVRQAPGRGLEWVSFISGRVFTNYTASVRGRFTVFREDDNTSVYLQMSRLRVEDTAVYYCARLRGIFRGPLKPLEYYFDLWGRGTLVTVSSASTKGPSVFPLAPSSKSTSGGTAALGCLVKDYFPEPVTVSWNSGALTSGVHTFPAVLQSSGLYSLSSVVTVPSSSLGTQTYICNVNHKPSNTKVDKKVEPKSCDKTHTCPPCPAPELLGGPSVFLFPPKPKDTLMISRTPEVTCVVVDVSHEDPEVKFNWYVDGVEVHNAKTKPREEQYNSTYRVVSVLTVLHQDWLNGKEYKCKVSNKALPAPIEKTISKAKGQPREPQVYTLPPSRDELTKNQVSLTCLVKGFYPSDIAVEWESNGQPENNYKTTPPVLDSDGSFFLYSKLTVDKSRWQQGNVFSCSVMHEALHNHYTQKSLSLSPGK

SEQ ID NO: 2 - protein, 219 aa, synthetic construct
  REGION 1..219: note = mAb637-IgG1 light chain
NFELTQPHSVSESPGKTVTISCTRSSGSIASNYVQWYQQRPGSSPTTVIYEDNQRPSGVPDRFSGSIDSSSNSASLTISGLKTEDEADYYCQSYDSNSGGRVFGGGTKLTVLRTVAAPSVFIFPPSDEQLKSGTASVVCLLNNFYPREAKVQWKVDNALQSGNSQESVTEQDSKDSTYSLSSTLTLSKADYEKHKVYACEVTHQGLSSPVTKSFNRGEC

SEQ ID NO: 3 - protein, 434 aa, synthetic construct
  REGION 1..434: note = mAb192 C IgG2/4 heavy chain
DIQMTQSPPSLSASLGDKVTITCQASQDINKYIAWYQQKPGKAPRQLIRYTSILVLGTPSRFSGSGSGRDFSFSISNVASEDIASYYCLQYGNLYTFGAGTKLEIKRSSASTKGPSVFPLAPCSRSTSESTAALGCLVKDYFPEPVTVSWNSGALTSGVHTFPAVLQSSGLYSLSSVVTVPSSNFGTQTYTCNVDHKPSNTKVDKTVERKCCVECPPCPAPPVAGPSVFLFPPKPKDTLMISRTPEVTCVVVDVSQEDPEVQFNWYVDGVEVHNAKTKPREEQFNSTYRVVSVLTVLHQDWLNGKEYKCKVSNKGLPSSIEKTISKAKGQPREPQVYTLPPSQEEMTKNQVSLTCLVKGFYPSDIAVEWESNGQPENYKTTPPVLDSDGSFFLYSRLTVDKSRWQEGNVFSCSVMHEALHNHYTQKSLSLSLGK

SEQ ID NO: 4 - protein, 224 aa, synthetic construct
  REGION 1..224: note = mAb192 C IgG2/4 light chain
QVQLLESGPGLVQPSQTLSLTCTVSGFSLTTNGVSWVRQPPGKGLEWIAAISSGGSPYYNSALKSRLSINRDTSKSQVFLKMNSLQTEDTAIYFCTREDGWNYFDYWGPGTMVTVSSASVAAPSVFIFPPSDEQLKSGTASVVCLLNNFYPREAKVQWKVDNALQSGNSQESVTEQDSKDSTYSLSSTLTLSKADYEKHKVYACEVTHQGLSSPVTKSFNRGEC

SEQ ID NO: 5 - protein, 446 aa, synthetic construct
  REGION 1..446: note = mAb192 BIgG2/4 heavy chain
DIQMTQSPPSLSASLGDKVTITCQASQDINKYIAWYQQKPGKAPRQLIRYTSILVLGTPSRFSGSGSGRDFSFSISNVASEDIASYYCLQYGNLYTFGAGTKLEIKRRTVAAPSVFIFPPSDEQLKSGTASVVCLLNNFYPREAKVQWKVDNALQSGNSQESVTEQDSKDSTYSLSSTLTLSKADYEKHKVYACEVTHQGLSSPVTKSFNRGECEPKSCDKTHTCPPCPAPELLGGPSVFLFPPKPKDTLMISRTPEVTCVVVDVSHEDPEVKFNWYVDGVEVHNAKTKPREEQYNSTYRVVSVLTVLHQDWLNGKEYKCKVSNKALPAPIEKTISKAKGQPREPQVYTLPPSRDELTKNQVSLTCLVKGFYPSDIAVEWESNGQPENNYKTTPPVLDSDGSFFLYSKLTVDKSRWQQGNVFSCSVMHEALHNHYTQKSLSLSPGK

SEQ ID NO: 6 - protein, 215 aa, synthetic construct
  REGION 1..215: note = mAb192 BIgG2/4 light chain
QVQLLESGPGLVQPSQTLSLTCTVSGFSLTTNGVSWVRQPPGKGLEWIAAISSGGSPYYNSALKSRLSINRDTSKSQVFLKMNSLQTEDTAIYFCTREDGWNYFDYWGPGTMVTVSSASTKGPSVFPLAPSSKSTSGGTAALGCLVKDYFPEPVTVSWNSGALTSGVHTFPAVLQSSGLYSLSSVVTVPSSSLGTQTYICNVNHKPSNTKVDKKV

SEQ ID NO: 7 - protein, 445 aa, synthetic construct
  REGION 1..445: note = rAb58 heavy chain
VQLVESGGGLVQPGGSLRLSCAASGFTFRGYAMNWVRQAPGKGLEWVASISGSGSITQYADSAKGRFTITRDNSKSTLYAHVSSLRADDTAVYYCAKGDYVFDYWGQGTLVTVSSASTKGPSVFPLAPSSKSTSGGTAALGCLVKDYFPEPVTVSWNSGALTSGVHTFPAVLQSSGLYSLSSVVTVPSSSLGTQTYICNVNHKPSNTKVDKKVEPKSCDKTHTCPPCPAPELLGGPSVFLFPPKPKDTLMISRTPEVTCVVVDVSHEDPEVKFNWYVDGVEVHNAKTKPREEQYNSTYRVVSVLTVLHQDWLNGKEYKCKVSNKALPAPIEKTISKAKGQPREPQVYTLPPSRDELTKNQVSLTCLVKGFYPSDIAVEWESNGQPENNYKTTPPVLDSDGSFFLYSKLTVDKSRWQQGNVFSCSVMHEALHNHYTQKSLSLSPGK

SEQ ID NO: 8 - protein, 217 aa, synthetic construct
  REGION 1..217: note = rAb58 light chain
DIQMTQSPSALSASVGDTVTITCRASQSIRSWLAWYQQKPGKAPKLLIYKASDLQSGVPSRFSGSGSGTDFTLTISGLQPDDFATYYCQHYNSYPYTFGQGTKVEIRRTVRTVAAPSVFIFPPSDEQLKSGTASVVCLLNNFYPREAKVQWKVDNALQSGNSQESVTEQDSKDSTYSLSSTLTLSKADYEKHKVYACEVTHQGLSSPVTKSFNRGEC

SEQ ID NO: 9 - protein, 435 aa, synthetic construct
  REGION 1..435: note = rAb53 C IgG2/4 heavy chain
EIVLTQSPGTLSLSPGERATLSCRASQTVRTNYLAWFQQKPGQAPRLLIFGASSRATGIPDRFSGSGSGTDFTLTISRLEPEDFAVYYCQQYGSSPWTFGQGTKVEIKSSASTKGPSVFPLAPCSRSTSESTAALGCLVKDYFPEPVTVSWNSGALTSGVHTFPAVLQSSGLYSLSSVVTVPSSNFGTQTYTCNVDHKPSNTKVDKTVERKCCVECPPCPAPPVAGPSVFLFPPKPKDTLMISRTPEVTCVVVDVSQEDPEVQFNWYVDGVEVHNAKTKPREEQFNSTYRVVSVLTVLHQDWLNGKEYKCKVSNKGLPSSIEKTISKAKGQPREPQVYTLPPSQEEMTKNQVSLTCLVKGFYPSDIAVEWESNGQPENYKTTPPVLDSDGSFFLYSKLTVDKSRWQEGNVFSCSVMHEALHNHYTQKSLSLSLGK

SEQ ID NO: 10 - protein, 231 aa, synthetic construct
  REGION 1..231: note = rAb53 C IgG2/4 light chain
QVQLQESGAGLVKPSETLSLTCTVSGGSISGHYWNWIRQPPGKGLEWIGRIHYSGRTNYNPSLKSRVTISVDTSKNQFSLKLSSVTAADTAVYYCARAEGRGWSAFYYYYMEVWGKGSTVSVSSASVAAPSVFIFPPSDEQLKSGTASVVCLLNNFYPREAKVQWKVDNALQSGNSQESVTEQDSKDSTYSLSSTLTLSKADYEKHKVYACEVTHQGLSSPVTKSFNRGEC

SEQ ID NO: 11 - protein, 450 aa, synthetic construct
  REGION 1..450: note = mAb35 rat IgG heavy chain
QVKLQESGPGLVQPSETLSLTCTVSGFSLTSYSVSWLRQPSGKGPEWMGRMWDDGGTVYNSGLKSRLSISRDTSKNQVFLKMNSLQTDDTGTYYCTRDERIRAINWFAYWGQGTLVTVSSASTKGPSVFPLAPSSKSTSGGTAALGCLVKDYFPEPVTVSWNSGALTSGVHTFPAVLQSSGLYSLSSVVTVPSSSLGTQTYICNVNHKPSNTKVDKKVEPKSCDKTHTCPPCPAPELLGGPSVFLFPPKPKDTLMISRTPEVTCVVVDVSHEDPEVKFNWYVDGVEVHNAKTKPREEQYNSTYRVVSVLTVLHQDWLNGKEYKCKVSNKALPAPIEKTISKAKGQPREPQVYTLPPSRDELTKNQVSLTCLVKGFYPSDIAVEWESNGQPENNYKTTPPVLDSDGSFFLYSKLTVDKSRWQQGNVFSCSVMHEALHNHYTQKSLSLSPGK

SEQ ID NO: 12 - protein, 213 aa, synthetic construct
  REGION 1..213: note = mAb35 rat IgG light chain
NIQLTQSPSLLTYLDDPNSTLTCKGSQNIDNYLAWYQQKLGEAPKLLIYKTNSLQTGIPSRFSGSGSGTDYTLTISSLHSEDELATYYCYQYINGYTFGTGTKLELRTVAAPSVFIFPPSDEQLKSGTASVVCLLNNFYPREAKVQWKVDNALQSGNSQESVTEQDSKDSTYSLSSTLTLSKADYEKHKVYACEVTHQGLSSPVTKSFNRGEC

SEQ ID NO: 13 - protein, 439 aa, synthetic construct
  REGION 1..439: note = mAb35 B heavy chain
DIVITQSPSLLSASVGDRVTLTCKGSQNIDNYLAWYQQKLGEAPKLLIYKTNSLQTGIPSRFSGSGSGTDYTLTISSLHSEDLATYYCYQYINGYTFGTGTKLELASVAAPSVFIFPPSDEQLKSGTASVVCLLNNFYPREAKVQWKVDNALQSGNSQESVTEQDSKDSTYSLSSTLTLSKADYEKHKVYACEVTHQGLSSPVTKSFNRGECERKCCVECPPCPAPPVAGPSVFLFPPKPKDTLMISRTPEVTCVVVDVSQEDPEVQFNWYVDGVEVHNAKTKPREEQFNSTYRVVSVLTVLHQDWLNGKEYKCKVSNKGLPSSIEKTISKAKGQPREPQVYTLPPSQEEMTKNQVSLTCLVKGFYPSDIAVEWESNGQPENYKTTPPVLDSDGSFFLYSKLTVDKSRWQEGNVFSCSVMHEALHNHYTQKSLSLSLGK

SEQ ID NO: 14 - protein, 218 aa, synthetic construct
  REGION 1..218: note = mAb35 B light chain
EVQLQESGPGLVQPSETLSLTCTVSGFSLTSYSVSWLRQPSGKGPEWMGRMWDDGGTVYNSGLKSRLSISRDTSKNQVFLKMNSLQTDDTGTYYCTRDERIRAINWFAYWGQGTLVTVSSASTKGPSVFPLAPCSRSTSESTAALGCLVKDYFPEPVTVSWNSGALTSGVHTFPAVLQSSGLYSLSSVVTVPSSNFGTQTYTCNVDHKPSNTKVDKTV

SEQ ID NO: 15 - protein, 432 aa, synthetic construct
  REGION 1..432: note = mAb35 C heavy chain
DIVITQSPSLLSASVGDRVTLTCKGSQNIDNYLAWYQQKLGEAPKLLIYKTNSLQTGIPSRFSGSGSGTDYTLTISSLHSEDLATYYCYQYINGYTFGTGTKLELSSASTKGPSVFPLAPCSRSTSESTAALGCLVKDYFPEPVTVSWNSGALTSGVHTFPAVLQSSGLYSLSSVVTVPSSNFGTQTYTCNVDHKPSNTKVDKTVERKCCVECPPCPAPPVAGPSVFLFPPKPKDTLMISRTPEVTCVVVDVSQEDPEVQFNWYVDGVEVHNAKTKPREEQFNSTYRVVSVLTVLHQDWLNGKEYKCKVSNKGLPSSIEKTISKAKGQPREPQVYTLPPSQEEMTKNQVSLTCLVKGFYPSDIAVEWESNGQPENYKTTPPVLDSDGSFFLYSKLTVDKSRWQEGNVFSCSVMHEALHNHYTQKSLSLSLGK

SEQ ID NO: 16 - protein, 227 aa, synthetic construct
  REGION 1..227: note = mAb35 C light chain
EVQLQESGPGLVQPSETLSLTCTVSGFSLTSYSVSWLRQPSGKGPEWMGRMWDDGGTVYNSGLKSRLSISRDTSKNQVFLKMNSLQTDDTGTYYCTRDERIRAINWFAYWGQGTLVTVSSASVAAPSVFIFPPSDEQLKSGTASVVCLLNNFYPREAKVQWKVDNALQSGNSQESVTEQDSKDSTYSLSSTLTLSKADYEKHKVYACEVTHQGLSSPVTKSFNRGEC

SEQ ID NO: 17 - protein, 446 aa, synthetic construct
  REGION 1..446: note = mAb637 B heavy chain
NFELTQPHSVSESPGKTVTISCTRSSGSIASNYVQWYQQRPGSSPTTVIYEDNQRPSGVPDRFSGSIDSSSNSASLTISGLKTEDEADYYCQSYDSNSGGRVFGGGTKLTVLRTVAAPSVFIFPPSDEQLKSGTASVVCLLNNFYPREAKVQWKVDNALQSGNSQESVTEQDSKDSTYSLSSTLTLSKADYEKHKVYACEVTHQGLSSPVTKSFNRGECERKCCVECPPCPAPPVAGPSVFLFPPKPKDTLMISRTPEVTCVVVDVSQEDPEVQFNWYVDGVEVHNAKTKPREEQFNSTYRVVSVLTVLHQDWLNGKEYKCKVSNKGLPSSIEKTISKAKGQPREPQVYTLPPSQEEMTKNQVSLTCLVKGFYPSDIAVEWESNGQPENYKTTPPVLDSDGSFFLYSRLTVDKSRWQEGNVFSCSVMHEALHNHYTQKSLSLSLGK

SEQ ID NO: 18 - protein, 224 aa, synthetic construct
  REGION 1..224: note = mAb637 B light chain
QVQLLESGGGLVKPGGSLRLSCAASGFKSTDYYMAWVRQAPGRGLEWVSFISGRVFTNYTASVRGRFTVFREDDNTSVYLQMSRLRVEDTAVYYCARLRGIFRGPLKPLEYYFDLWGRGTLVTVSSASTKGPSVFPLAPCSRSTSESTAALGCLVKDYFPEPVTVSWNSGALTSGVHTFPAVLQSSGLYSLSSVVTVPSSNFGTQTYTCNVDHKPSNTKVDKTV

SEQ ID NO: 19 - protein, 437 aa, synthetic construct
  REGION 1..437: note = mAb637 C heavy chain
NFELTQPHSVSESPGKTVTISCTRSSGSIASNYVQWYQQRPGSSPTTVIYEDNQRPSGVPDRFSGSIDSSSNSASLTISGLKTEDEADYYCQSYDSNSGGRVFGGGTKLTVLASTKGPSVFPLAPCSRSTSESTAALGCLVKDYFPEPVTVSWNSGALTSGVHTFPAVLQSSGLYSLSSVVTVPSSNFGTQTYTCNVDHKPSNTKVDKTVERKCCVECPPCPAPPVAGPSVFLFPPKPKDTLMISRTPEVTCVVVDVSQEDPEVQFNWYVDGVEVHNAKTKPREEQFNSTYRVVSVLTVLHQDWLNGKEYKCKVSNKGLPSSIEKTISKAKGQPREPQVYTLPPSQEEMTKNQVSLTCLVKGFYPSDIAVEWESNGQPENYKTTPPVLDSDGSFFLYSRLTVDKSRWQEGNVFSCSVMHEALHNHYTQKSLSLSLGK

SEQ ID NO: 20 - protein, 233 aa, synthetic construct
  REGION 1..233: note = mAb637 C light chain
QVQLLESGGGLVKPGGSLRLSCAASGFKSTDYYMAWVRQAPGRGLEWVSFISGRVFTNYTASVRGRFTVFREDDNTSVYLQMSRLRVEDTAVYYCARLRGIFRGPLKPLEYYFDLWGRGTLVTVSSRTVAAPSVFIFPPSDEQLKSGTASVVCLLNNFYPREAKVQWKVDNALQSGNSQESVTEQDSKDSTYSLSSTLTLSKADYEKHKVYACEVTHQGLSSPVTKSFNRGEC

SEQ ID NO: 21 - protein, 8 aa, synthetic construct
  REGION 1..8: note = mAb637 VH CDR1
GFKSTDYY

SEQ ID NO: 22 - protein, 6 aa, synthetic construct
  REGION 1..6: note = mAb637 VH CDR2
SGRVFT

SEQ ID NO: 23 - protein, 20 aa, synthetic construct
  REGION 1..20: note = mAb637 VH CDR3
ARLRGIFRGPLKPLEYYFDL

SEQ ID NO: 24 - protein, 7 aa, synthetic construct
  REGION 1..7: note = mAb637 VL CDR1
GSIASNY

SEQ ID NO: 25 - skipped

SEQ ID NO: 26 - protein, 11 aa, synthetic construct
  REGION 1..11: note = mAb637 VL CDR3
QSYDSNSGGRV

SEQ ID NO: 27 - protein, 8 aa, synthetic construct
  REGION 1..8: note = mAb192 VH CDR1
GFSLTTNG

SEQ ID NO: 28 - protein, 7 aa, synthetic construct
  REGION 1..7: note = mAb192 VH CDR2
ISSGGSP

SEQ ID NO: 29 - protein, 11 aa, synthetic construct
  REGION 1..11: note = mAb192 VH CDR3
TREDGWNYFDY

SEQ ID NO: 30 - protein, 11 aa, synthetic construct
  REGION 1..11: note = mAb192 VL CDR1
QASQDINKYIA

SEQ ID NO: 31 - protein, 5 aa, synthetic construct
  REGION 1..5: note = mAb192 VL CDR2
YTSIL

SEQ ID NO: 32 - protein, 8 aa, synthetic construct
  REGION 1..8: note = mAb192 VL CDR3
LQYGNLYT

SEQ ID NO: 33 - protein, 8 aa, synthetic construct
  REGION 1..8: note = mAb35 VH CDR1
GFSLTSYS

SEQ ID NO: 34 - protein, 7 aa, synthetic construct
  REGION 1..7: note = mAb35 VH CDR2
MWDDGGT

SEQ ID NO: 35 - protein, 14 aa, synthetic construct
  REGION 1..14: note = mAb35 VH CDR3
TRDERIRAINWFAY

SEQ ID NO: 36 - protein, 6 aa, synthetic construct
  REGION 1..6: note = mAb35 VL CDR1
QNIDNY

SEQ ID NO: 37 - skipped

SEQ ID NO: 38 - protein, 5 aa, synthetic construct
  REGION 1..5: note = mAb35 VL CDR3
YQYIN

SEQ ID NO: 39 - protein, 8 aa, synthetic construct
  REGION 1..8: note = rAb53 VH CDR1
GGSISGHY

SEQ ID NO: 40 - protein, 7 aa, synthetic construct
  REGION 1..7: note = rAb53 VH CDR2
IHYSGRT

SEQ ID NO: 41 - protein, 18 aa, synthetic construct
  REGION 1..18: note = rAb53 VH CDR3
ARAEGRGWSAFYYYYMEV

SEQ ID NO: 42 - protein, 7 aa, synthetic construct
  REGION 1..7: note = rAb53 VL CDR1
QTVRTNY

SEQ ID NO: 43 - skipped

SEQ ID NO: 44 - protein, 9 aa, synthetic construct
  REGION 1..9: note = rAb53 VL CDR3
QQYGSSPWT

SEQ ID NO: 45 - protein, 447 aa, synthetic construct
  REGION 1..447: note = mAb192 IgG1 heavy chain
QVQLLESGPGLVQPSQTLSLTCTVSGFSLTTNGVSWVRQPPGKGLEWIAAISSGGSPYYNSALKSRLSINRDTSKSQVFLKMNSLQTEDTAIYFCTREDGWNYFDYWGPGTMVTVSSASTKGPSVFPLAPSSKSTSGGTAALGCLVKDYFPEPVTVSWNSGALTSGVHTFPAVLQSSGLYSLSSVVTVPSSSLGTQTYICNVNHKPSNTKVDKKVEPKSCDKTHTCPPCPAPELLGGPSVFLFPPKPKDTLMISRTPEVTCVVVDVSHEDPEVKFNWYVDGVEVHNAKTKPREEQYNSTYRVVSVLTVLHQDWLNGKEYKCKVSNKALPAPIEKTISKAKGQPREPQVYTLPPSRDELTKNQVSLTCLVKGFYPSDIAVEWESNGQPENNYKTTPPVLDSDGSFFLYSKLTVDKSRWQQGNVFSCSVMHEALHNHYTQKSLSLSPGK

SEQ ID NO: 46 - protein, 214 aa, synthetic construct
  REGION 1..214: note = mAb192 IgG1 light chain
DIQMTQSPPSLSASLGDKVTITCQASQDINKYIAWYQQKPGKAPRQLIRYTSILVLGTPSRFSGSGSGRDFSFSISNVASEDIASYYCLQYGNLYTFGAGTKLEIKRRTVAAPSVFIFPPSDEQLKSGTASVVCLLNNFYPREAKVQWKVDNALQSGNSQESVTEQDSKDSTYSLSSTLTLSKADYEKHKVYACEVTHQGLSSPVTKSFNRGEC

SEQ ID NO: 47 - protein, 454 aa, synthetic construct
  REGION 1..454: note = rAb53 IgG1 heavy chain
QVQLQESGAGLVKPSETLSLTCTVSGGSISGHYWNWIRQPPGKGLEWIGRIHYSGRTNYNPSLKSRVTISVDTSKNQFSLKLSSVTAADTAVYYCARAEGRGWSAFYYYYMEVWGKGSTVSVSSASTKGPSVFPLAPSSKSTSGGTAALGCLVKDYFPEPVTVSWNSGALTSGVHTFPAVLQSSGLYSLSSVVTVPSSSLGTQTYICNVNHKPSNTKVDKKVEPKSCDKTHTCPPCPAPELLGGPSVFLFPPKPKDTLMISRTPEVTCVVVDVSHEDPEVKFNWYVDGVEVHNAKTKPREEQYNSTYRVVSVLTVLHQDWLNGKEYKCKVSNKALPAPIEKTISKAKGQPREPQVYTLPPSRDELTKNQVSLTCLVKGFYPSDIAVEWESNGQPENNYKTTPPVLDSDGSFFLYSKLTVDKSRWQQGNVFSCSVMHEALHNHYTQKSLSLSPGK

SEQ ID NO: 48 - protein, 215 aa, synthetic construct
  REGION 1..215: note = rAb53 IgG1 light chain
EIVLTQSPGTLSLSPGERATLSCRASQTVRTNYLAWFQQKPGQAPRLLIFGASSRATGIPDRFSGSGSGTDFTLTISRLEPEDFAVYYCQQYGSSPWTFGQGTKVEIKRTVAAPSVFIFPPSDEQLKSGTASVVCLLNNFYPREAKVQWKVDNALQSGNSQESVTEQDSKDSTYSLSSTLTLSKADYEKHKVYACEVTHQGLSSPVTKSFNRGEC

SEQ ID NO: 49 - protein, 126 aa, synthetic construct
  REGION 1..126: note = mAb637-IgG1 VH
QVQLLESGGGLVKPGGSLRLSCAASGFKSTDYYMAWVRQAPGRGLEWVSFISGRVFTNYTASVRGRFTVFREDDNTSVYLQMSRLRVEDTAVYYCARLRGIFRGPLKPLEYYFDLWGRGTLVTVSS

SEQ ID NO: 50 - protein, 112 aa, synthetic construct
  REGION 1..112: note = mAb637-IgG1 VL
NFELTQPHSVSESPGKTVTISCTRSSGSIASNYVQWYQQRPGSSPTTVIYEDNQRPSGVPDRFSGSIDSSSNSASLTISGLKTEDEADYYCQSYDSNSGGRVFGGGTKLTVL

SEQ ID NO: 51 - protein, 115 aa, synthetic construct
  REGION 1..115: note = rAb58 VH
VQLVESGGGLVQPGGSLRLSCAASGFTFRGYAMNWVRQAPGKGLEWVASISGSGSITQYADSAKGRFTITRDNSKSTLYAHVSSLRADDTAVYYCAKGDYVFDYWGQGTLVTVSS

SEQ ID NO: 52 - protein, 110 aa, synthetic construct
  REGION 1..110: note = rAb58 VL
DIQMTQSPSALSASVGDTVTITCRASQSIRSWLAWYQQKPGKAPKLLIYKASDLQSGVPSRFSGSGSGTDFTLTISGLQPDDFATYYCQHYNSYPYTFGQGTKVEIRRTV

SEQ ID NO: 53 - protein, 117 aa, synthetic construct
  REGION 1..117: note = mAb192 IgG1 VH
QVQLLESGPGLVQPSQTLSLTCTVSGFSLTTNGVSWVRQPPGKGLEWIAAISSGGSPYYNSALKSRLSINRDTSKSQVFLKMNSLQTEDTAIYFCTREDGWNYFDYWGPGTMVTVSS

SEQ ID NO: 54 - protein, 107 aa, synthetic construct
  REGION 1..107: note = mAb192 IgG1 VL
DIQMTQSPPSLSASLGDKVTITCQASQDINKYIAWYQQKPGKAPRQLIRYTSILVLGTPSRFSGSGSGRDFSFSISNVASEDIASYYCLQYGNLYTFGAGTKLEIKR

SEQ ID NO: 55 - protein, 124 aa, synthetic construct
  REGION 1..124: note = rAb53 C IgG2/4 VH
QVQLQESGAGLVKPSETLSLTCTVSGGSISGHYWNWIRQPPGKGLEWIGRIHYSGRTNYNPSLKSRVTISVDTSKNQFSLKLSSVTAADTAVYYCARAEGRGWSAFYYYYMEVWGKGSTVSVSS

SEQ ID NO: 56 - protein, 108 aa, synthetic construct
  REGION 1..108: note = rAb53 C IgG2/4 VL
EIVLTQSPGTLSLSPGERATLSCRASQTVRTNYLAWFQQKPGQAPRLLIFGASSRATGIPDRFSGSGSGTDFTLTISRLEPEDFAVYYCQQYGSSPWTFGQGTKVEIK

SEQ ID NO: 57 - protein, 120 aa, synthetic construct
  REGION 1..120: note = mAb35 rat IgG VH
QVKLQESGPGLVQPSETLSLTCTVSGFSLTSYSVSWLRQPSGKGPEWMGRMWDDGGTVYNSGLKSRLSISRDTSKNQVFLKMNSLQTDDTGTYYCTRDERIRAINWFAYWGQGTLVTVSS

SEQ ID NO: 58 - protein, 106 aa, synthetic construct
  REGION 1..106: note = mAb35 rat IgG VL
NIQLTQSPSLLTYLDDPNSTLTCKGSQNIDNYLAWYQQKLGEAPKLLIYKTNSLQTGIPSRFSGSGSGTDYTLTISSLHSEDELATYYCYQYINGYTFGTGTKLEL

SEQ ID NO: 59 - protein, 105 aa, synthetic construct
  REGION 1..105: note = mAb35 C VH
DIVITQSPSLLSASVGDRVTLTCKGSQNIDNYLAWYQQKLGEAPKLLIYKTNSLQTGIPSRFSGSGSGTDYTLTISSLHSEDLATYYCYQYINGYTFGTGTKLEL

SEQ ID NO: 60 - protein, 120 aa, synthetic construct
  REGION 1..120: note = mAb35 C VL
EVQLQESGPGLVQPSETLSLTCTVSGFSLTSYSVSWLRQPSGKGPEWMGRMWDDGGTVYNSGLKSRLSISRDTSKNQVFLKMNSLQTDDTGTYYCTRDERIRAINWFAYWGQGTLVTVSS

SEQ ID NO: 61 - protein, 126 aa, synthetic construct; identical to SEQ ID NO: 49
  REGION 1..126: note = mAb637 B VH

SEQ ID NO: 62 - protein, 111 aa, synthetic construct
  REGION 1..111: note = mAb637 B VL
NFELTQPHSVSESPGKTVTISCTRSSGSIASNYVQWYQQRPGSSPTTVIYEDNQRPSGVPDRFSGSIDSSSNSASLTISGLKTEDEADYYCQSYDSNSGGRVFGGGTKLTV

SEQ ID NO: 63 - protein, 124 aa, synthetic construct; identical to SEQ ID NO: 55
  REGION 1..124: note = rAb53 IgG1 VH

SEQ ID NO: 64 - protein, 108 aa, synthetic construct; identical to SEQ ID NO: 56
  REGION 1..108: note = rAb53 IgG1 VL

SEQ ID NO: 65 - protein, 442 aa, synthetic construct
  REGION 1..442: note = mAb192 IgG2/4 heavy chain
QVQLLESGPGLVQPSQTLSLTCTVSGFSLTTNGVSWVRQPPGKGLEWIAAISSGGSPYYNSALKSRLSINRDTSKSQVFLKMNSLQTEDTAIYFCTREDGWNYFDYWGPGTMVTVSSASTKGPSVFPLAPCSRSTSESTAALGCLVKDYFPEPVTVSWNSGALTSGVHTFPAVLQSSGLYSLSSVVTVPSSNFGTQTYTCNVDHKPSNTKVDKTVERKCCVECPPCPAPPVAGPSVFLFPPKPKDTLMISRTPEVTCVVVDVSQEDPEVQFNWYVDGVEVHNAKTKPREEQFNSTYRVVSVLTVLHQDWLNGKEYKCKVSNKGLPSSIEKTISKAKGQPREPQVYTLPPSQEEMTKNQVSLTCLVKGFYPSDIAVEWESNGQPENYKTTPPVLDSDGSFFLYSRLTVDKSRWQEGNVFSCSVMHEALHNHYTQKSLSLSLGK

SEQ ID NO: 66 - protein, 214 aa, synthetic construct; identical to SEQ ID NO: 46
  REGION 1..214: note = mAb192 IgG2/4 light chain

SEQ ID NO: 67 - protein, 117 aa, synthetic construct; identical to SEQ ID NO: 53
  REGION 1..117: note = mAb192 IgG2/4 VH

SEQ ID NO: 68 - protein, 107 aa, synthetic construct; identical to SEQ ID NO: 54
  REGION 1..107: note = mAb192 IgG2/4 VL

SEQ ID NO: 69 - protein, 439 aa, synthetic construct
  REGION 1..439: note = mAb192 C IgG1 heavy chain
DIQMTQSPPSLSASLGDKVTITCQASQDINKYIAWYQQKPGKAPRQLIRYTSILVLGTPSRFSGSGSGRDFSFSISNVASEDIASYYCLQYGNLYTFGAGTKLEIKRSSASTKGPSVFPLAPSSKSTSGGTAALGCLVKDYFPEPVTVSWNSGALTSGVHTFPAVLQSSGLYSLSSVVTVPSSSLGTQTYICNVNHKPSNTKVDKKVEPKSCDKTHTCPPCPAPELLGGPSVFLFPPKPKDTLMISRTPEVTCVVVDVSHEDPEVKFNWYVDGVEVHNAKTKPREEQYNSTYRVVSVLTVLHQDWLNGKEYKCKVSNKALPAPIEKTISKAKGQPREPQVYTLPPSRDELTKNQVSLTCLVKGFYPSDIAVEWESNGQPENNYKTTPPVLDSDGSFFLYSKLTVDKSRWQQGNVFSCSVMHEALHNHYTQKSLSLSPGK

SEQ ID NO: 70 - protein, 224 aa, synthetic construct; identical to SEQ ID NO: 4
  REGION 1..224: note = mAb192 C IgG1 light chain

SEQ ID NO: 71 - protein, 436 aa, synthetic construct
  REGION 1..436: note = mAb192 C IgG4 heavy chain
DIQMTQSPPSLSASLGDKVTITCQASQDINKYIAWYQQKPGKAPRQLIRYTSILVLGTPSRFSGSGSGRDFSFSISNVASEDIASYYCLQYGNLYTFGAGTKLEIKRSSASTKGPSVFPLAPCSRSTSESTAALGCLVKDYFPEPVTVSWNSGALTSGVHTFPAVLQSSGLYSLSSVVTVPSSSLGTKTYTCNVDHKPSNTKVDKRVESKYGPPCPPCPAPEFEGGPSVFLFPPKPKDTLMISRTPEVTCVVVDVSQEDPEVQFNWYVDGVEVHNAKTKPREEQFNSTYRVVSVLTVLHQDWLNGKEYKCKVSNKGLPSSIEKTISKAKGQPREPQVYTLPPSQEEMTKNQVSLTCLVKGFYPSDIAVEWESNGQPENNYKTTPPVLDSDGSFFLYSRLTVDKSRWQEGNVFSCSVMHEALHNHYTQKSLSLSLGK

SEQ ID NO: 72 - protein, 224 aa, synthetic construct; identical to SEQ ID NO: 4
  REGION 1..224: note = mAb192 C IgG4 light chain

SEQ ID NO: 73 - protein, 450 aa, synthetic construct
  REGION 1..450: note = mAb35 humanized antibody heavy chain
EVQLQESGPGLVQPSETLSLTCTVSGFSLTSYSVSWLRQPSGKGPEWMGRMWDDGGTVYNSGLKSRLSISRDTSKNQVFLKMNSLQTDDTGTYYCTRDERIRAINWFAYWGQGTLVTVSSASTKGPSVFPLAPSSKSTSGGTAALGCLVKDYFPEPVTVSWNSGALTSGVHTFPAVLQSSGLYSLSSVVTVPSSSLGTQTYICNVNHKPSNTKVDKKVEPKSCDKTHTCPPCPAPELLGGPSVFLFPPKPKDTLMISRTPEVTCVVVDVSHEDPEVKFNWYVDGVEVHNAKTKPREEQYNSTYRVVSVLTVLHQDWLNGKEYKCKVSNKALPAPIEKTISKAKGQPREPQVYTLPPSRDELTKNQVSLTCLVKGFYPSDIAVEWESNGQPENNYKTTPPVLDSDGSFFLYSKLTVDKSRWQQGNVFSCSVMHEALHNHYTQKSLSLSPGK

SEQ ID NO: 74 - protein, 212 aa, synthetic construct
  REGION 1..212: note = mAb35 humanized antibody light chain
DIVITQSPSLLSASVGDRVTLTCKGSQNIDNYLAWYQQKLGEAPKLLIYKTNSLQTGIPSRFSGSGSGTDYTLTISSLHSEDLATYYCYQYINGYTFGTGTKLELRTVAAPSVFIFPPSDEQLKSGTASVVCLLNNFYPREAKVQWKVDNALQSGNSQESVTEQDSKDSTYSLSSTLTLSKADYEKHKVYACEVTHQGLSSPVTKSFNRGEC

SEQ ID NO: 75 - protein, 120 aa, synthetic construct; identical to SEQ ID NO: 60
  REGION 1..120: note = mAb35 humanized antibody VH

SEQ ID NO: 76 - protein, 105 aa, synthetic construct; identical to SEQ ID NO: 59
  REGION 1..105: note = mAb35 humanized antibody VL